European Patent Specification EP 3 768 711 B1, published May 3, 2023. Title: ANTI-CD137 ANTIBODIES FOR COMBINATION WITH ANTI-PD-L1 ANTIBODIES. Applicant: Eli Lilly and Company. The sequence listing filed with the application follows.

SEQUENCE LISTING (26 sequences)

SEQ ID NO: 1 - protein, 255 aa, Homo sapiens
MGNSCYNIVATLLLVLNFERTRSLQDPCSNCPAGTFCDNNRNQICSPCPPNSFSSAGGQRTCDICRQCKGVFRTRKECSSTSNAECDCTPGFHCLGAGCSMCEQDCKQGQELTKKGCKDCCFGTFNDQKRGICRPWTNCSLDGKSVLVNGTKERDVVCGPSPADLSPGASSVTPPAPAREPGHSPQIISFFLALTSTALLFLLFFLTLRFSVVKRGRKKLLYIFKQPFMRPVQTTQEEDGCSCRFPEEEEGGCEL

SEQ ID NO: 2 - protein, 13 aa, Artificial Sequence
  synthetic peptide
KASGGTFSSYAIS

SEQ ID NO: 3 - protein, 17 aa, Artificial Sequence
  synthetic peptide
GIIPIFGTANYAQKFQG

SEQ ID NO: 4 - protein, 15 aa, Artificial Sequence
  synthetic peptide
ARDLMTTAPGTYFDL

SEQ ID NO: 5 - protein, 11 aa, Artificial Sequence
  synthetic peptide
QASQDIGNSLG

SEQ ID NO: 6 - protein, 8 aa, Artificial Sequence
  synthetic peptide
FDASDLET

SEQ ID NO: 7 - protein, 9 aa, Artificial Sequence
  synthetic peptide
QQGNSFPLT

SEQ ID NO: 8 - protein, 120 aa, Artificial Sequence
  synthetic peptide
QVQLVQSGAEVKKPGSSVKVSCKASGGTFSSYAISWVRQAPGQGLEWMGGIIPIFGTANYAQKFQGRVTITADESTSTAYMELSSLRSEDTAVYYCARDLMTTAPGTYFDLWGRGTLVTV

SEQ ID NO: 9 - protein, 107 aa, Artificial Sequence
  synthetic sequence
AIRMTQSPPSLSASVGDRVTITCQASQDIGNSLGWYQQKPGKAPKLVIFDASDLETGVPSRFSGSGSGTDFSLTISSLQPEDFATYYCQQGNSFPLTFGQGTRLEIK

SEQ ID NO: 10 - protein, 452 aa, Artificial Sequence
  synthetic sequence
QVQLVQSGAEVKKPGSSVKVSCKASGGTFSSYAISWVRQAPGQGLEWMGGIIPIFGTANYAQKFQGRVTITADESTSTAYMELSSLRSEDTAVYYCARDLMTTAPGTYFDLWGRGTLVTVSSASTKGPSVFPLAPSSKSTSGGTAALGCLVKDYFPEPVTVSWNSGALTSGVHTFPAVLQSSGLYSLSSVVTVPSSSLGTQTYICNVNHKPSNTKVDKRVEPKSCDKTHTCPPCPAPEAEGAPSVFLFPPKPKDTLMISRTPEVTCVVVDVSHEDPEVKFNWYVDGVEVHNAKTKPREEQYNSTYRVVSVLTVLHQDWLNGKEYKCKVSNKALPSSIEKTISKAKGQPREPQVYTLPPSREEMTKNQVSLTCLVKGFYPSDIAVEWESNGQPENNYKTTPPVLDSDGSFFLYSKLTVDKSRWQQGNVFSCSVMHEALHNHYTQKSLSLSPGK

SEQ ID NO: 11 - protein, 214 aa, Artificial Sequence
  synthetic sequence
AIRMTQSPPSLSASVGDRVTITCQASQDIGNSLGWYQQKPGKAPKLVIFDASDLETGVPSRFSGSGSGTDFSLTISSLQPEDFATYYCQQGNSFPLTFGQGTRLEIKRTVAAPSVFIFPPSDEQLKSGTASVVCLLNNFYPREAKVQWKVDNALQSGNSQESVTEQDSKDSTYSLSSTLTLSKADYEKHKVYACEVTHQGLSSPVTKSFNRGEC

SEQ ID NO: 12 - protein, 106 aa, Artificial Sequence
  synthetic sequence
IRMTQSPPSLSASVGDRVTITCQASQDIGNSLGWYQQKPGKAPKLVIFDASDLETGVPSRFSGSGSGTDFSLTISSLQPEDFATYYCQQGNSFPLTFGQGTRLEIK

SEQ ID NO: 13 - protein, 213 aa, Artificial Sequence
  synthetic sequence
IRMTQSPPSLSASVGDRVTITCQASQDIGNSLGWYQQKPGKAPKLVIFDASDLETGVPSRFSGSGSGTDFSLTISSLQPEDFATYYCQQGNSFPLTFGQGTRLEIKRTVAAPSVFIFPPSDEQLKSGTASVVCLLNNFYPREAKVQWKVDNALQSGNSQESVTEQDSKDSTYSLSSTLTLSKADYEKHKVYACEVTHQGLSSPVTKSFNRGEC

SEQ ID NO: 14 - DNA, 1359 bp, Artificial Sequence
  synthetic sequence
caggtgcagctggtgcagtctggggctgaggtgaagaagcctgggtcctcggtgaaggtctcctgcaaggcttctggaggcaccttcagcagctatgctatcagctgggtgcgacaggcccctggacaagggcttgagtggatgggagggatcatccctatctttggtacagcaaactacgcacagaagttccagggcagagtcacgattaccgcggacgaatccacgagcacagcctacatggagctgagcagcctgagatctgaggacacggccgtgtattactgtgcgagagatctgatgactacggcccctgggacgtacttcgatctctggggccgtggcaccctggtcactgtctcctcagctagcaccaagggcccatcggtcttccccctggcaccctcctccaagagcacctctgggggcacagcggccctgggctgcctggtcaaggactacttccccgaaccggtgacggtgtcgtggaactcaggcgcactgaccagcggcgtgcacaccttcccggctgtcctacagtcctcaggactctactccctcagcagcgtggtgaccgtgccctccagcagcttgggcacccagacctacatctgcaacgtgaatcacaagcccagcaacaccaaggtggacaagagagttgagcccaaatcttgtgacaaaactcacacatgcccaccgtgcccagcacctgaagccgagggggcaccgtcagtcttcctcttccccccaaaacccaaggacaccctcatgatctcccggacccctgaggtcacatgcgtggtggtggacgtgagccacgaagaccctgaggtcaagttcaactggtatgtggacggcgtggaggtgcataatgccaagacaaagccgcgggaggagcagtacaacagcacgtaccgtgtggtcagcgtcctcaccgtcctgcaccaagactggctgaatggcaaggagtacaagtgcaaggtctccaacaaagccctcccatcctccatcgagaaaaccatctccaaagccaaagggcagccccgagaaccacaggtgtacaccctgcccccatcccgggaggagatgaccaagaaccaagtcagcctgacctgcctggtcaaaggcttctatcccagcgacatcgccgtggagtgggagagcaatgggcagccggagaacaactacaagaccacgcctcccgtgctggactccgacggctccttcttcctctattccaagctcaccgtggacaagagcaggtggcagcaggggaacgtcttctcatgctccgtgatgcatgaggctctgcacaaccactacacgcagaagagcctctccctgtctccgggcaaatga

SEQ ID NO: 15 - DNA, 645 bp, Artificial Sequence
  synthetic sequence
atgaggctgctgcctctgctggccctcctggccctgtggggcccagacccagccagagccgccatccggatgacccagtctccaccctccctgtctgcatctgtaggagacagagtcaccatcacttgccaggcgagtcaggacattggcaactctttaggttggtatcagcagaaaccagggaaagcccctaaactcgtgatcttcgatgcatcagatctggaaacaggggtcccatcaaggttcagtggcagtggatctggcacagatttcagtctcaccatcagcagcctgcagcctgaggattttgcaacttactattgtcaacagggtaacagtttcccgctcaccttcggccaagggacacgactggagattaaacgaactgcctctgttgtgtgcctgctgaataacttctatcccagagaggccaaagtacagtggaaggtggataacgccctccaatcgggtaactcccaggagagtgtcacagagcaggacagcaaggacagcacctacagcctcagcagcaccctgacgctgagcaaagcagactacgagaaacacaaagtctacgcctgcgaagtcacccatcagggcctgagctcgcccgtcacaaagagcttcaacaggggagagtgttag

SEQ ID NO: 16 - DNA, 702 bp, Artificial Sequence
  synthetic sequence
atggagacagacacactcctgctatgggtactgctgctctgggttccaggctccaccggcatccggatgacccagtctccaccctccctgtctgcatctgtaggagacagagtcaccatcacttgccaggcgagtcaggacattggcaactctttaggttggtatcagcagaaaccagggaaagcccctaaactcgtgatcttcgatgcatcagatctggaaacaggggtcccatcaaggttcagtggcagtggatctggcacagatttcagtctcaccatcagcagcctgcagcctgaggattttgcaacttactattgtcaacagggtaacagtttcccgctcaccttcggccaagggacacgactggagattaaacgaactgtggccgcaccatctgtcttcatcttcccgccatctgatgagcagttgaaatctggaactgcctctgttgtgtgcctgctgaataacttctatcccagagaggccaaagtacagtggaaggtggataacgccctccaatcgggtaactcccaggagagtgtcacagagcaggacagcaaggacagcacctacagcctcagcagcaccctgacgctgagcaaagcagactacgagaaacacaaagtctacgcctgcgaagtcacccatcagggcctgagctcgcccgtcacaaagagcttcaacaggggagagtgttag

SEQ ID NO: 17 - DNA, 705 bp, Artificial Sequence
  synthetic sequence
atggagacagacacactcctgctatgggtactgctgctctgggttccaggctccaccggcgccatccggatgacccagtctccaccctccctgtctgcatctgtaggagacagagtcaccatcacttgccaggcgagtcaggacattggcaactctttaggttggtatcagcagaaaccagggaaagcccctaaactcgtgatcttcgatgcatcagatctggaaacaggggtcccatcaaggttcagtggcagtggatctggcacagatttcagtctcaccatcagcagcctgcagcctgaggattttgcaacttactattgtcaacagggtaacagtttcccgctcaccttcggccaagggacacgactggagattaaacgaactgtggctgcaccatctgtcttcatcttcccgccatctgatgagcagttgaaatctggaactgcctctgttgtgtgcctgctgaataacttctatcccagagaggccaaagtacagtggaaggtggataacgccctccaatcgggtaactcccaggagagtgtcacagagcaggacagcaaggacagcacctacagcctcagcagcaccctgacgctgagcaaagcagactacgagaaacacaaagtctacgcctgcgaagtcacccatcagggcctgagctcgcccgtcacaaagagcttcaacaggggagagtgttag

SEQ ID NO: 18 - protein, 448 aa, Artificial Sequence
  synthetic sequence
QVQLQQWGAGLLKPSETLSLTCAVYGGSFSGYYWSWIRQSPEKGLEWIGEINHGGYVTYNPSLESRVTISVDTSKNQFSLKLSSVTAADTAVYYCARDYGPGNYDWYFDLWGRGTLVTVSSASTKGPSVFPLAPCSRSTSESTAALGCLVKDYFPEPVTVSWNSGALTSGVHTFPAVLQSSGLYSLSSVVTVPSSSLGTKTYTCNVDHKPSNTKVDKRVESKYGPPCPPCPAPEFLGGPSVFLFPPKPKDTLMISRTPEVTCVVVDVSQEDPEVQFNWYVDGVEVHNAKTKPREEQFNSTYRVVSVLTVLHQDWLNGKEYKCKVSNKGLPSSIEKTISKAKGQPREPQVYTLPPSQEEMTKNQVSLTCLVKGFYPSDIAVEWESNGQPENNYKTTPPVLDSDGSFFLYSRLTVDKSRWQEGNVFSCSVMHEALHNHYTQKSLSLSLGK

SEQ ID NO: 19 - protein, 216 aa, Artificial Sequence
  synthetic sequence
EIVLTQSPATLSLSPGERATLSCRASQSVSSYLAWYQQKPGQAPRLLIYDASNRATGIPARFSGSGSGTDFTLTISSLEPEDFAVYYCQQRSNWPPALTFGGGTKVEIKRTVAAPSVFIFPPSDEQLKSGTASVVCLLNNFYPREAKVQWKVDNALQSGNSQESVTEQDSKDSTYSLSSTLTLSKADYEKHKVYACEVTHQGLSSPVTKSFNRGEC

SEQ ID NO: 20 - protein, 676 aa, Artificial Sequence
  synthetic sequence
EVQLVQSGAEVKKPGESLRISCKGSGYSFSTYWISWVRQMPGKGLEWMGKIYPGDSYTNYSPSFQGQVTISADKSISTAYLQWSSLKASDTAMYYCARGYGIFDYWGQGTLVTVSSASTKGPSVFPLAPCSRSTSESTAALGCLVKDYFPEPVTVSWNSGALTSGVHTFPAVLQSSGLYSLSSVVTVPSSNFGTQTYTCNVDHKPSNTKVDKTVERKCCVECPPCPAPPVAGPSVFLFPPKPKDTLMISRTPEVTCVVVDVSHEDPEVQFNWYVDGVEVHNAKTKPREEQFNSTFRVVSVLTVVHQDWLNGKEYKCKVSNKGLPAPIEKTISKTKGQPREPQVYTLPPSREEMTKNQVSLTCLVKGFYPSDIAVEWESNGQPEMETDTLLLWVLLLWVPGSTGAIRMTQSPPSLSASVGDRVTITCQASQDIGNSLGWYQQKPGKAPKLVIFDASDLETGVPSRFSGSGSGTDFSLTISSLQPEDFATYYCQQGNSFPLTFGQGTRLEIKRTVAAPSVFIFPPSDEQLKSGTASVVCLLNNFYPREAKVQWKVDNALQSGNSQESVTEQDSKDSTYSLSSTLTLSKADYEKHKVYACEVTHQGLSSPVTKSFNRGECNNYKTTPPMLDSDGSFFLYSKLTVDKSRWQQGNVFSCSVMHEALHNHYTQKSLSLSPGK

SEQ ID NO: 21 - protein, 214 aa, Artificial Sequence
  synthetic sequence
SYELTQPPSVSVSPGQTASITCSGDNIGDQYAHWYQQKPGQSPVLVIYQDKNRPSGIPERFSGSNSGNTATLTISGTQAMDEADYYCATYTGFGSLAVFGGGTKLTVLGQPKAAPSVTLFPPSSEELQANKATLVCLISDFYPGAVTVAWKADSSPVKAGVETTTPSKQSNNKYAASSYLSLTPEQWKSHRSYSCQVTHEGSTVEKTVAPTECS

SEQ ID NO: 22 - protein, 123 aa, Artificial Sequence
  synthetic sequence
QVQLVQSGAEVKKPGSSVKVSCKASGGTFSSYAISWVRQAPGQGLEWMGGIIPIFGTANYAQKFQGRVTITADKSTSTAYMELSSLRSEDTAVYYCARSPDYSPYYYYGMDVWGQGTTVTVSS

SEQ ID NO: 23 - protein, 111 aa, Artificial Sequence
  synthetic sequence
QSVLTQPPSASGTPGQRVTISCSGSSSNIGSNTVNWYQQLPGTAPKLLIYGNSNRPSGVPDRFSGSKSGTSASLAISGLQSEDEADYYCQSYDSSLSGSVFGGGIKLTVLG

SEQ ID NO: 24 - protein, 453 aa, Artificial Sequence
  synthetic sequence
QVQLVQSGAEVKKPGSSVKVSCKASGGTFSSYAISWVRQAPGQGLEWMGGIIPIFGTANYAQKFQGRVTITADKSTSTAYMELSSLRSEDTAVYYCARSPDYSPYYYYGMDVWGQGTTVTVSSASTKGPSVFPLAPSSKSTSGGTAALGCLVKDYFPEPVTVSWNSGALTSGVHTFPAVLQSSGLYSLSSVVTVPSSSLGTQTYICNVNHKPSNTKVDKRVEPKSCDKTHTCPPCPAPEAEGAPSVFLFPPKPKDTLMISRTPEVTCVVVDVSHEDPEVKFNWYVDGVEVHNAKTKPREEQYNSTYRVVSVLTVLHQDWLNGKEYKCKVSNKALPSSIEKTISKAKGQPREPQVYTLPPSREEMTKNQVSLTCLVKGFYPSDIAVEWESNGQPENNYKTTPPVLDSDGSFFLYSKLTVDKSRWQQGNVFSCSVMHEALHNHYTQKSLSLSPGK

SEQ ID NO: 25 - protein, 216 aa, Artificial Sequence
  synthetic sequence
QSVLTQPPSASGTPGQRVTISCSGSSSNIGSNTVNWYQQLPGTAPKLLIYGNSNRPSGVPDRFSGSKSGTSASLAISGLQSEDEADYYCQSYDSSLSGSVFGGGIKLTVLGQPKAAPSVTLFPPSSEELQANKATLVCLISDFYPGAVTVAWKADSSPVKAGVETTTPSKQSNNKYAASSYLSLTPEQWKSHRSYSCQVTHEGSTVEKTVAPAECS

SEQ ID NO: 26 - protein, 290 aa, Artificial Sequence
  synthetic sequence
MRIFAVFIFMTYWHLLNAFTVTVPKDLYVVEYGSNMTIECKFPVEKQLDLAALIVYWEMEDKNIIQFVHGEEDLKVQHSSYRQRARLLKDQLSLGNAALQITDVKLQDAGVYRCMISYGGADYKRITVKVNAPYNKINQRILVVDPVTSEHELTCQAEGYPKAEVIWTSSDHQVLSGKTTTTNSKREEKLFNVTSTLRINTTTNEIFYCTFRRLDPEENHTAELVIPELPLAHPPNERTHLVILGAILLCLGVALTFIFRLRKGRMMDVKKCGIQDTNSKKQSDTHLEET